European Patent Application EP 4 796 642 A1, published August 26, 2026. Title: 用于生产重组腺相关病毒载体的方法及包装/生产细胞. Applicant: 深圳市深研生物科技有限公司. The sequence listing filed with the application follows.

SEQUENCE LISTING (13 sequences)

SEQ ID NO: 1 - DNA, 585 bp, synthetic construct
  source 1..585: mol_type = other DNA
atggcacccaaaaagaagctgcagctgccgccgccacccacggacgaggaggaatactgggacagtcaggcagaggaggttttggacgaggaggaggaggacatgatggaagactgggagagcctagacgaggaagcttccgaggtcgaagaggtgtcagacgaaacaccgtcaccctcggtcgcattcccctcgccggcgccccagaaatcggcaaccggttccagcatggctacaacctccgctcctcaggcgccgccggcactgcccgttcgccgacccaaccgtagatgggacaccactggaaccagggccggtaagtccaagcagccgccgccgttagcccaagagcaacaacagcgccaaggctaccgctcatggcgcgggcacaagaacgccatagttgcttgcttgcaagactgtgggggcaacatctccttcgcccgccgctttcttctctaccatcacggcgtggccttcccccgtaacatcctgcattactaccgtcatctctacagcccatactgcaccggcggcagcggcagcaacagcagcggccacacagaagcaaaggcgaccggatag

SEQ ID NO: 2 - protein, 194 aa, synthetic construct
MAPKKKLQLPPPPTDEEEYWDSQAEEVLDEEEEDMMEDWESLDEEASEVEEVSDETPSPSVAFPSPAPQKSATGSSMATTSAPQAPPALPVRRPNRRWDTTGTRAGKSKQPPPLAQEQQQRQGYRSWRGHKNAIVACLQDCGGNISFARRFLLYHHGVAFPRNILHYYRHLYSPYCTGGSGSNSSGHTEAKATG

SEQ ID NO: 3 - DNA, 684 bp, synthetic construct
  source 1..684: mol_type = other DNA
atggcacccaaaaagaagctgcagctgccgccgccacccacggacgaggaggaatactgggacagtcaggcagaggaggttttggacgaggaggaggaggacatgatggaagactgggagagcctagacgaggaagcttccgaggtcgaagaggtgtcagacgaaacaccgtcaccctcggtcgcattcccctcgccggcgccccagaaatcggcaaccggttccagcatggctacaacctccgctcctcaggcgccgccggcactgcccgttcgccgacccaaccgtagatgggacaccactggaaccagggccgcccatactgcaccggcggcagcggcagcaacagcagcggccacacagaagcaaaggcgaccggatagcaagactctgacaaagcccaagaaatccacagcggcggcagcagcaggaggaggagcgctgcgtctggcgcccaacgaacccgtatcgacccgcgagcttagaaacaggatttttcccactctgtatgctatatttcaacagagcaggggccaagaacaagagctgaaaataaaaaacaggtctctgcgatccctcacccgcagctgcctgtatcacaaaagcgaagatcagcttcggcgcacgctggaagacgcggaggctctcttcagtaaatactgcgcgctgactcttaaggactag

SEQ ID NO: 4 - protein, 227 aa, synthetic construct
MAPKKKLQLPPPPTDEEEYWDSQAEEVLDEEEEDMMEDWESLDEEASEVEEVSDETPSPSVAFPSPAPQKSATGSSMATTSAPQAPPALPVRRPNRRWDTTGTRAAHTAPAAAAATAAATQKQRRPDSKTLTKPKKSTAAAAAGGGALRLAPNEPVSTRELRNRIFPTLYAIFQQSRGQEQELKIKNRSLRSLTRSCLYHKSEDQLRRTLEDAEALFSKYCALTLKD

SEQ ID NO: 5 - DNA, 886 bp, synthetic construct
  source 1..886: mol_type = other DNA
atggcacccaaaaagaagctgcagctgccgccgccacccacggacgaggaggaatactgggacagtcaggcagaggaggttttggacgaggaggaggaggacatgatggaagactgggagagcctagacgaggaagcttccgaggtcgaagaggtgtcagacgaaacaccgtcaccctcggtcgcattcccctcgccggcgccccagaaatcggcaaccggttccagcatggctacaacctccgctcctcaggcgccgccggcactgcccgttcgccgacccaaccgtagatgggacaccactggaaccagggccggtaagtccaagcagccgccgccgttagcccaagagcaacaacagcgccaaggctaccgctcatggcgcgggcacaagaacgccatagttgcttgcttgcaagactgtgggggcaacatctccttcgcccgccgctttcttctctaccatcacggcgtggccttcccccgtaacatcctgcattactaccgtcatctctacagcccatactgcaccggcggcagcggcagcaacagcagcggccacacagaagcaaaggcgaccggatagcaagactctgacaaagcccaagaaatccacagcggcggcagcagcaggaggaggagcgctgcgtctggcgcccaacgaacccgtatcgacccgcgagcttagaaacaggatttttcccactctgtatgctatatttcaacagagcaggggccaagaacaagagctgaaaataaaaaacaggtctctgcgatccctcacccgcagctgcctgtatcacaaaagcgaagatcagcttcggcgcacgctggaagacgcggaggctctcttcagtaaatactgcgcgctgactcttaaggactag

SEQ ID NO: 6 - DNA, 2649 bp, synthetic construct
  source 1..2649: mol_type = other DNA
atggcggcggccggcggggagcgccagctagacggacagaaacccggcccgccgcaccttcagcaacccggggaccgaccagccgttccagggagggccgaggcctttttaaattttacgtctatgcacggggtgcagccaatccttaagcgcatccgagagctctcgcaacaacagctcgacggagcgcaagtgccccgtctgcagtggttccgggacgtggcggccttagagtcccccgcaggcctgcccctcagggagtttccgttcgcggtgtatcttatcaccggcaacgctggctccggaaagagcacgtgcgtgcagacaatcaacgaggtcttggactgtgtggtgacgggcgccacgcgcattgcggcccaaaacatgtacgccaaactctcgggcgcctttctcagccgacccatcaacaccatctttcatgaatttgggtttcgcgggaatcacgtccaggcccaactgggacagtacccgtacaccctgaccagcaaccccgcctcgctggaggacctgcagcgacgagatctgacgtactactgggaggtgattttggacctcacgaagcgcgccctggccgcctccgggggcgaggagttgcggaacgagtttcgcgccctggccgccctggaacggaccctggggttggccgagggcgccctgacgcggttggccccggccacccacggggcgctgccggcctttacccgcagcaacgtgatcgtcatcgacgaggccgggctccttgggcgtcacctcctcacggccgtggtgtattgctggtggatgattaacgccctgtaccacaccccccagtacgcggcccgcctgcggcccgtgttggtgtgtgtgggctcgccgacgcagacggcgtccctggagtcgaccttcgagcaccagaaactgcggtgttccgtccgccagagcgagaacgtgctcacgtacctcatctgcaaccgcacgctgcgcgagtacgcccgcctctcgtatagctgggccatttttattaacaacaaacggtgcgtcgagcacgagttcggtaacctcatgaaggtgctggagtacggcctgcccatcaccgaggagcacatgcagttcgtggatcgcttcgtcgtcccggaaaactacatcaccaaccccgccaacctccccggctggacgcggctgttctcctcccacaaagaggtgagcgcgtacatggccaagctccacgcctacctgaaggtgacccgtgagggggagttcgtcgtgttcaccctccccgtgcttacgttcgtgtcggtcaaggagtttgacgaataccgacggctgacacaccagcccggcctgactattgaaaagtggctcacggccaacgccagccgcatcaccaactactcgcagagccaggaccaggacgcggggcacatgcgctgcgaggtgcacagcaaacagcagctggtcgtggcccgcaacgacgtcacttacgtcctcaacagccagatcgcggtgaccgcgcgcctgcgaaaactggtttttgggtttagtgggacgttccgggccttcgaggcagtgttgcgtgacgacagctttgtaaagactcagggggagacttcggtggagtttgcctacaggttcctgtcgcggctcatatttagcgggcttatctccttttacaactttctgcagcgcccgggcctggatgcgacccagaggaccctcgcgtacgcccgcatgggagaactaacggcggagattctgtctctgcgccccaaatcttcgggggtgccgacgcaggcgtcggtaatggccgacgcaggcgcccccggcgagcgtgcgtttgattttaagcaactggggccgcgggacgggggcccggacgattttcccgacgacgacctcgacgttattttcgcggggctggacgaacaacagctcgacgtgttttactgccactacacccccggggaaccggagaccaccgccgccgttcacacccagtttgcgctgctgaagcgggccttcctcgggagattccgaatcctccaagagctcttcggggaggcatttgaagtcgccccctttagcacgtacgtggacaacgttatcttccggggctgcgagatgctgaccggctcgccgcgcggggggctgatgtccgtcgccctgcagacggacaattatacgctcatgggatacacgtacacacgggtgtttgcctttgcggacgagctgcggaggcggcacgcgacggccaacgtggccgagttactggaagaggcccccctgccttacgtggtcttgcgggaccaacacggcttcatgtccgtcgtcaacaccaacatcagcgagtttgtcgagtccattgactctacggagctggccatggccataaacgccgactacggcatcagctccaagcttgccatgaccatcacgcgctcccagggccttagcctggacaaggtcgccatctgctttacgcccggcaacctgcgcctcaacagcgcgtacgtggccatgtcccgcaccacctcctccgaattccttcgcatgaacttaaatccgctccgggagcgccacgagcgcgatgacgtcattagtgagcacatactatcggctctgcgcgatccgaacgtggtcattgtctattaa

SEQ ID NO: 7 - protein, 882 aa, synthetic construct
MAAAGGERQLDGQKPGPPHLQQPGDRPAVPGRAEAFLNFTSMHGVQPILKRIRELSQQQLDGAQVPRLQWFRDVAALESPAGLPLREFPFAVYLITGNAGSGKSTCVQTINEVLDCVVTGATRIAAQNMYAKLSGAFLSRPINTIFHEFGFRGNHVQAQLGQYPYTLTSNPASLEDLQRRDLTYYWEVILDLTKRALAASGGEELRNEFRALAALERTLGLAEGALTRLAPATHGALPAFTRSNVIVIDEAGLLGRHLLTAVVYCWWMINALYHTPQYAARLRPVLVCVGSPTQTASLESTFEHQKLRCSVRQSENVLTYLICNRTLREYARLSYSWAIFINNKRCVEHEFGNLMKVLEYGLPITEEHMQFVDRFVVPENYITNPANLPGWTRLFSSHKEVSAYMAKLHAYLKVTREGEFVVFTLPVLTFVSVKEFDEYRRLTHQPGLTIEKWLTANASRITNYSQSQDQDAGHMRCEVHSKQQLVVARNDVTYVLNSQIAVTARLRKLVFGFSGTFRAFEAVLRDDSFVKTQGETSVEFAYRFLSRLIFSGLISFYNFLQRPGLDATQRTLAYARMGELTAEILSLRPKSSGVPTQASVMADAGAPGERAFDFKQLGPRDGGPDDFPDDDLDVIFAGLDEQQLDVFYCHYTPGEPETTAAVHTQFALLKRAFLGRFRILQELFGEAFEVAPFSTYVDNVIFRGCEMLTGSPRGGLMSVALQTDNYTLMGYTYTRVFAFADELRRRHATANVAELLEEAPLPYVVLRDQHGFMSVVNTNISEFVESIDSTELAMAINADYGISSKLAMTITRSQGLSLDKVAICFTPGNLRLNSAYVAMSRTTSSEFLRMNLNPLRERHERDDVISEHILSALRDPNVVIVY

SEQ ID NO: 8 - DNA, 2253 bp, synthetic construct
  source 1..2253: mol_type = other DNA
atggacaccgcagatatcgtgtgggtggaggagagcgtcagcgccattaccctttacgcggtatggctgcccccccgcgctcgcgagtacttccacgccctggtgtattttgtatgtcgcaacgccgcaggggagggtcgcgcgcgctttgcggaggtctccgtcaccgcgacggagctgcgggatttctacggctccgcggacgtctccgtccaggccgtcgtggcggccgcccgcgccgcgacgacgccggccgcctccccgctggagcccctggagaacccgactctgtggcgggcgctgtacgcgtgcgtcctggcggccctggagcgccagaccgggccggtggccctgttcgccccgctgcgtatcggctcggacccacgcacgggactggtggtgaaagttgagagagcgtcgtggggcccgcccgccgcccctcgcgccgctctcctggtcgcggaggccaacattgacatcgaccctatggccctggcggcgcgcgttgccgagcatcccgacgcgcggctggcgtgggcgcgcctggcggccattcgcgacaccccccagtgcgcgtccgccgcttcgctgaccgttaacatcaccaccggaaccgcgctatttgcgcgcgaataccagactcttgcgtttccgccgatcaagaaggagggcgcgttcggggacctggtcgaggtgtgcgaggtgggcctgcggccacgcgggcacccgcaacgagtcacggcacgggtgctgctgccccgcgattacgactactttgtaagcgccggcgagaagttctccgcgccggcgctcgtcgcccttttccggcagtggcataccacggtccacgccgcccccggggccctggcccccgtctttgcctttctggggcccgagtttgaggtccgggggggacccgtcccgtactttgccgtcctggggtttccgggttggcccacgttcaccgtgccggccacggccgagtcggcacgggacctggtgcgcggggccgcggccgcttacgccgcgctcctgggggcctggcccgcggtgggggccagggtcgtcctccccccgcgagcctggcccggcgtggcctcggcggcagccggatgcctcctgcccgcggtgcgggaggcggtggcgcggtggcatcccgccactaaaatcatccaactgttagacccgcccgcggccgtcgggcccgtctggacggcgcggttttgcttccccggacttcgcgcccagctcctggcggccctggccgacctcggggggagcgggctggcggacccccacggccggacgggcctagcaagactggacgcgctggtggtggccgctccctcagagccctgggccggggccgtcttggagcgcctggtcccggacacgtgcgacgcctgccctgcgctgcggcagctcctgggtggggtaatggccgccgtctgcctgcagatcgaggagacggccagctcggtgaagttcgcggtctgcgggggcgatgggggtgcgttctggggtgtctttaacgtggacccccaagacgcggatgcggcttccggggtgatcgaggacgcccggcgggccatcgagacggccgtgggagccgtgcttagggccaacggcctccggctgcggcacccactgtgcctggccctcgagggcgtctacacccacgcagtcgcctggaaccaggcgggagtgtggttctggaactcccgcgacaacactgaccatcttgggggatttcctctccgcgggcccgcgtacaccacggcggccggggtcgtacgcgacacgctgcgacgggtcctgggcctgacaacggcaggcgtgccggaggaggacgcactcacggcccggggccttatggaggacgcctgcgaccgccttatcgtggacgcgtttaataaacggttggacgcggagtactggagcgttcgggtgtccccctttgaggctagcgaccccttgccccccactgccttccgcggcggcgccttgctggacgcagagcactactggcggcgcgtcgtgcgtgtctgtcccggaggcggggagtcggtcggcgtccccgtcgatctatacccgcggccccttgtgctcccccccgtggactgcgctcatcacctgcgcgaaatcctgcgcgagattgagttggtgtttaccggggtgctggcgggagtatggggagagggggggaagtttgtgtatccctttgacgacaagatgtcgtttctgtttgcctga

SEQ ID NO: 9 - protein, 750 aa, synthetic construct
MDTADIVWVEESVSAITLYAVWLPPRAREYFHALVYFVCRNAAGEGRARFAEVSVTATELRDFYGSADVSVQAVVAAARAATTPAASPLEPLENPTLWRALYACVLAALERQTGPVALFAPLRIGSDPRTGLVVKVERASWGPPAAPRAALLVAEANIDIDPMALAARVAEHPDARLAWARLAAIRDTPQCASAASLTVNITTGTALFAREYQTLAFPPIKKEGAFGDLVEVCEVGLRPRGHPQRVTARVLLPRDYDYFVSAGEKFSAPALVALFRQWHTTVHAAPGALAPVFAFLGPEFEVRGGPVPYFAVLGFPGWPTFTVPATAESARDLVRGAAAAYAALLGAWPAVGARVVLPPRAWPGVASAAAGCLLPAVREAVARWHPATKIIQLLDPPAAVGPVWTARFCFPGLRAQLLAALADLGGSGLADPHGRTGLARLDALVVAAPSEPWAGAVLERLVPDTCDACPALRQLLGGVMAAVCLQIEETASSVKFAVCGGDGGAFWGVFNVDPQDADAASGVIEDARRAIETAVGAVLRANGLRLRHPLCLALEGVYTHAVAWNQAGVWFWNSRDNTDHLGGFPLRGPAYTTAAGVVRDTLRRVLGLTTAGVPEEDALTARGLMEDACDRLIVDAFNKRLDAEYWSVRVSPFEASDPLPPTAFRGGALLDAEHYWRRVVRVCPGGGESVGVPVDLYPRPLVLPPVDCAHHLREILREIELVFTGVLAGVWGEGGKFVYPFDDKMSFLFA

SEQ ID NO: 10 - DNA, 3591 bp, synthetic construct
  source 1..3591: mol_type = other DNA
atggagacaaagcccaagacggcaaccaccatcaaggtcccccccgggcccctgggatacgtgtacgctcgcgcgtgtccgtccgaaggcatcgagcttctggcgttactgtcggcgcgcagcggcgatgccgacgtcgccgtggcgcccctggtcgtgggcctgaccgtggagagcggctttgaggccaacgtagccgtggtcgtgggttctcgcacgacggggctcgggggtaccgcggtgtccctgaaactgacgccatcgcactacagctcgtccgtgtacgtctttcacggcggccggcacctggaccccagcacccaggccccaaacctgacgcgactctgcgagcgggcacgccgccattttggcttttcggactacaccccccggcccggcgacctcaaacacgagacgacgggggaggcgctgtgtgagcgcctcggcctggacccggaccgcgccctcctgtatctggtcgttaccgagggcttcaaggaggccgtgtgcatcaacaacacctttctgcacctgggaggctcggacaaggtaaccataggcggggcggaggtgcaccgcatacccgtgtatccgttgcagctgttcatgccggattttagccgggtcatcgccgagccgttcaacgccaaccaccgatcgatcggggagaattttacctacccgcttccgttttttaaccgccccctcaaccgcctcctgttcgaggcggtcgtgggacccgccgccgtggcactgcgatgccgaaacgtggacgccgtggcccgcgcggccgcccacctggcgtttgacgaaaaccacgagggcgccgccctccccgccgacattacgttcacggccttcgaagccagccagggtaagaccccgcggggtgggcgcgacggcggcggcaagggcccggcgggcgggttcgaacagcgcctggcctccgtcatggccggagacgccgccctggccctcgagtctatcgtgtcgatggccgtcttcgacgagccgcccaccgacatctccgcgtggccgctgtgcgagggccaggacacggccgcggcccgcgccaacgccgtcggggcgtacctggcgcgcgccgcgggactcgtgggggccatggtatttagcaccaactcggccctccatctcaccgaggtggacgacgccggtccggcggacccaaaggaccacagcaaaccctccttttaccgcttcttcctcgtgcccgggacccacgtggcggccaacccacaggtggaccgcgagggacacgtggtgcccgggttcgagggtcggcccaccgcgcccctcgtcggcggaacccaggaatttgccggcgagcacctggccatgctgtgtgggttttccccggcgctgctggccaagatgctgttttacctggagcgctgcgacggcggcgtgatcgtcgggcgccaggagatggacgtgtttcgatacgtcgcggactccaaccagaccgacgtgccctgcaacctgtgcaccttcgacacgcgccacgcctgcgtacacacgacgctcatgcgcctccgggcgcgccatcccaagttcgccagcgccgcccgcggagccatcggcgtcttcgggaccatgaacagcatgtacagcgactgcgacgtgctgggaaactacgccgccttctcggccctgaagcgcgcggacggatccgagaccgcccggaccatcatgcaggagacgtaccgcgcggcgaccgagcgcgtcatggccgaactcgagaccctgcagtacgtggaccaggcggtccccacggccatggggcggctggagaccatcatcaccaaccgcgaggccctgcatacggtggtgaacaacgtcaggcaggtcgtggaccgcgaggtggagcagctgatgcgcaacctggtggaggggaggaacttcaagtttcgcgacggtctgggcgaggccaaccacgccatgtccctgacgctggacccgtacgcgtgcgggccatgccccctgcttcagcttctcgggcggcgatccaacctcgccgtgtatcaggacctggccctgagccagtgccacggggtgttcgccgggcagtcggtcgaggggcgcaactttcgcaatcaattccaaccggtgctgcggcggcgcgtgatggacatgtttaacaacgggtttctgtcggccaaaacgctgacggtcgcgctctcggagggggcggctatctgcgcccccagcctaacggccggccagacggcccccgccgagagcagcttcgagggcgacgttgcccgcgtgaccctggggtttcccaaggagctgcgcgtcaagagccgcgtgttgttcgcgggcgcgagcgccaacgcgtccgaggccgccaaggcgcgggtcgccagcctccagagcgcctaccagaagcccgacaagcgcgtggacatcctcctcggaccgctgggctttctgctgaagcagttccacgcggccatcttccccaacggcaagcccccggggtccaaccagccgaacccgcagtggttctggacggccctccaacgcaaccagcttcccgcccggctcctgtcgcgcgaggacatcgagaccatcgcgttcattaaaaagttttccctggactacggcgcgataaactttattaacctggcccccaacaacgtgagcgagctggcgatgtactacatggcaaaccagattctgcggtactgcgatcactcgacatacttcatcaacaccctcacggccatcatcgcggggtcccgccgtccccccagcgtgcaggcggcggccgcgtggtccgcgcagggcggggcgggcctggaggccggggcccgcgcgctgatggacgccgtggacgcgcatccgggcgcgtggacgtccatgttcgccagctgcaacctgctgcggcccgtcatggcggcgcgccccatggtcgtgttggggttgagcatcagcaaatactacggcatggccggcaacgaccgtgtgtttcaggccgggaactgggccagcctgatgggcggcaaaaacgcgtgcccgctccttatttttgaccgcacccgcaagttcgtcctggcctgtccccgggccgggtttgtgtgcgcggcctcgaacctcggcggcggagcgcacgaaagctcgctgtgcgagcagctccggggcattatctccgagggcggggcggccgtcgccagtagcgtgttcgtggcgaccgtgaaaagcctggggccccgcacccagcagctgcagatcgaggactggctggcgctcctggaggacgagtacctaagcgaggagatgatggagctgaccgcgcgtgccctggagcgcggcaacggcgagtggtcgacggacgcggccctggaggtggcgcacgaggccgaggccctagtcagccaactcggcaacgccggggaggtgtttaactttggggattttggctgcgaggacgacaacgcgacgccgttcggcggcccgggggccccgggaccggcatttgccggccgcaaacgggcgttccacggggatgacccgtttggggaggggccccccgacaaaaagggagacctgacgttggatatgctgtga

SEQ ID NO: 11 - protein, 1196 aa, synthetic construct
METKPKTATTIKVPPGPLGYVYARACPSEGIELLALLSARSGDADVAVAPLVVGLTVESGFEANVAVVVGSRTTGLGGTAVSLKLTPSHYSSSVYVFHGGRHLDPSTQAPNLTRLCERARRHFGFSDYTPRPGDLKHETTGEALCERLGLDPDRALLYLVVTEGFKEAVCINNTFLHLGGSDKVTIGGAEVHRIPVYPLQLFMPDFSRVIAEPFNANHRSIGENFTYPLPFFNRPLNRLLFEAVVGPAAVALRCRNVDAVARAAAHLAFDENHEGAALPADITFTAFEASQGKTPRGGRDGGGKGPAGGFEQRLASVMAGDAALALESIVSMAVFDEPPTDISAWPLCEGQDTAAARANAVGAYLARAAGLVGAMVFSTNSALHLTEVDDAGPADPKDHSKPSFYRFFLVPGTHVAANPQVDREGHVVPGFEGRPTAPLVGGTQEFAGEHLAMLCGFSPALLAKMLFYLERCDGGVIVGRQEMDVFRYVADSNQTDVPCNLCTFDTRHACVHTTLMRLRARHPKFASAARGAIGVFGTMNSMYSDCDVLGNYAAFSALKRADGSETARTIMQETYRAATERVMAELETLQYVDQAVPTAMGRLETIITNREALHTVVNNVRQVVDREVEQLMRNLVEGRNFKFRDGLGEANHAMSLTLDPYACGPCPLLQLLGRRSNLAVYQDLALSQCHGVFAGQSVEGRNFRNQFQPVLRRRVMDMFNNGFLSAKTLTVALSEGAAICAPSLTAGQTAPAESSFEGDVARVTLGFPKELRVKSRVLFAGASANASEAAKARVASLQSAYQKPDKRVDILLGPLGFLLKQFHAAIFPNGKPPGSNQPNPQWFWTALQRNQLPARLLSREDIETIAFIKKFSLDYGAINFINLAPNNVSELAMYYMANQILRYCDHSTYFINTLTAIIAGSRRPPSVQAAAAWSAQGGAGLEAGARALMDAVDAHPGAWTSMFASCNLLRPVMAARPMVVLGLSISKYYGMAGNDRVFQAGNWASLMGGKNACPLLIFDRTRKFVLACPRAGFVCAASNLGGGAHESSLCEQLRGIISEGGAAVASSVFVATVKSLGPRTQQLQIEDWLALLEDEYLSEEMMELTARALERGNGEWSTDAALEVAHEAEALVSQLGNAGEVFNFGDFGCEDDNATPFGGPGAPGPAFAGRKRAFHGDDPFGEGPPDKKGDLTLDML

SEQ ID NO: 12 - DNA, 3177 bp, synthetic construct
  source 1..3177: mol_type = other DNA
atggggcaggaagacgggaaccgcggggagaggcgggcggccgggactcccgtggaggtgaccgcgctttatgcgaccgacgggtgcgttattacctcttcgatcgccctcctcacaaactctctactgggggccgagccggtttatatattcagctacgacgcatacacgcacgatggccgtgccgacgggcccacggagcaagacaggttcgaagagagtcgggcgctctaccaagcgtcgggcgggctaaatggcgactccttccgagtaaccttttgtttattggggacggaagtgggtgggacccaccaggcccgcgggcgaacccgacccatgttcgtctgtcgcttcgagcgagcggacgacgtcgccgcgctacaggacgccctggcgcacgggaccccgctacaaccggaccacatcgccgccaccctggacgcggaggccacgttcgcgctgcatgcgaacatgatcctggctctcaccgtggccgtcaacaacgccagcccccgcaccggacgcgacgccgccgcggcgcagtatgatcagggcgcgtccctacgctcgctcgtggggcgcacgtccctgggacaacgcggccttaccacgctatacgtccaccacgaggcgcgcgtgctggccgcgtaccgcagggcgtattatggaagcgcgcagagtcccttctggtttcttagcaaattcgggcctgacgaaaaaagcctggtgctcaccactcggtactacctgcttcaggcccagcgtctggggggcgcgggggccacgtacgacctgcaggccatcaaggacatctgcgccacctacgcgattccccacgccccccgccccgacaccgtcagcgccgcgtccctgacctcgtttgccgccatcacgcggttctgttgcacgagccagtacgcccgcggggccgcggcggccgggtttccgctttacgtggagcgccgtattgcggccgacgtccgcgagaccagtgcgctggagaagttcataacccacgatcgcagttgcctgcgcgtgtccgaccgtgaattcattacgtacatttacctggcccattttgagtgtttcagccccccgcgcctagccacgcatcttcgggccgtgacgacccaggaccccaaccccgcggccaacacggagcagccctcgcccctgggcagggaggccgtggaacaatttttttgccacgtgcgcgcccaactgaatatcggggagtacgtcaaacacaacgtgaccccccgggagaccgtcctggatggcgatacggccaaggcctacctgcgcgctcgcacgtacgcgcccggggccctgacgcccgcccccgcgtattgcggggccgtggactccgccaccaaaatgatggggcgtttggcggacgccgaaaagctcctggtcccccgcgggtggcccgcgtttgcgcccgccagtcccggggaggatacggcgggcggcacgccgcccccacagacctgcggaatcgtcaagcgcctcctgagactggccgccacggaacaacaggacaccacgcccccggcgatcgcggcgcttatccgtaatgcggcggtgcagactcccctgcccgtctaccggatatccatggtccccacgggacaggcatttgccgcgctggcctgggacgactgggcccgcataacgcgggacgctcgcctggccgaagcggtcgtgtccgccgaagcggcggcgcaccccgaccacggcgcgctgggcaggcggctcacggatcgcatccgcgcccagggccccgtgatgccccctggcggcctggatgccggggggcagatgtacgtgaatcgcaacgagatatttaacggcgcgctggcaatcacaaacatcatcctggatctcgacatcgccctgaaggagcccgtcccctttcgccggctccacgaggccctgggccactttaggcgcggggctctggcggcggttcagctcctgtttcccgcggcccgcgtggaccccgacgcatatccctgttattttttcaaaagcgcatgtcggcccggcccggcgtccgtgggttccggcagcggactcggcaacgacgacgacggggactggtttccctgctacgacgacgccggtgatgaggagtgggcggaggacccgggcgccatggacacatcccacgatcccccggacgacgaggttgcctactttgacctgtgccacgaagtcggccccacggcggaacctcgcgaaacggattcgcccgtgtgttcctgcaccgacaagatcggactgcgggtgtgcatgcccgtccccgccccgtacgtcgtccacggttctctaacgatgcggggggtggcacgggtcatccagcaggcggtgctgttggaccgagattttgtggaggccatcgggagctacgtaaaaaacttcctgttgatcgatacgggggtgtacgcccacggccacagcctgcgtttgccgtattttgccaaaatcgcccccgacgggcctgcgtgcggaaggctgctgccagtgtttgtgatcccccccgcctgcaaagacgttccggcgtttgtcgccgcgcacgccgacccgcggcgcttccattttcacgccccgcccacctatctcgcttccccccgggagatccgtgtcctgcacagcctgggtggggactatgtgagcttctttgaaaggaaggcgtcccgcaacgcgctggaacactttgggcgacgcgagaccctgacggaggtcctgggtcggtacaacgtacagccggatgcgggggggaccgtcgaggggttcgcatcggaactgctggggcggatagtcgcgtgcatcgaaacccactttcccgaacacgccggcgaatatcaggccgtatccgtccggcgggccgtcagtaaggacgactgggtcctcctacagctagtccccgttcgcggtaccctgcagcaaagcctgtcgtgtctgcgctttaagcacggccgggcgagtcgcgccacggcgcggacattcgtcgcgctgagcgtcggggccaacaaccgcctgtgcgtgtccttgtgtcagcagtgctttgccgccaaatgcgacagcaaccgcctgcacacgctgtttaccattgacgccggcacgccatgctcgccgtccgttccctgcagcacctctcaaccgtcgtcttga

SEQ ID NO: 13 - protein, 1058 aa, synthetic construct
MGQEDGNRGERRAAGTPVEVTALYATDGCVITSSIALLTNSLLGAEPVYIFSYDAYTHDGRADGPTEQDRFEESRALYQASGGLNGDSFRVTFCLLGTEVGGTHQARGRTRPMFVCRFERADDVAALQDALAHGTPLQPDHIAATLDAEATFALHANMILALTVAVNNASPRTGRDAAAAQYDQGASLRSLVGRTSLGQRGLTTLYVHHEARVLAAYRRAYYGSAQSPFWFLSKFGPDEKSLVLTTRYYLLQAQRLGGAGATYDLQAIKDICATYAIPHAPRPDTVSAASLTSFAAITRFCCTSQYARGAAAAGFPLYVERRIAADVRETSALEKFITHDRSCLRVSDREFITYIYLAHFECFSPPRLATHLRAVTTQDPNPAANTEQPSPLGREAVEQFFCHVRAQLNIGEYVKHNVTPRETVLDGDTAKAYLRARTYAPGALTPAPAYCGAVDSATKMMGRLADAEKLLVPRGWPAFAPASPGEDTAGGTPPPQTCGIVKRLLRLAATEQQDTTPPAIAALIRNAAVQTPLPVYRISMVPTGQAFAALAWDDWARITRDARLAEAVVSAEAAAHPDHGALGRRLTDRIRAQGPVMPPGGLDAGGQMYVNRNEIFNGALAITNIILDLDIALKEPVPFRRLHEALGHFRRGALAAVQLLFPAARVDPDAYPCYFFKSACRPGPASVGSGSGLGNDDDGDWFPCYDDAGDEEWAEDPGAMDTSHDPPDDEVAYFDLCHEVGPTAEPRETDSPVCSCTDKIGLRVCMPVPAPYVVHGSLTMRGVARVIQQAVLLDRDFVEAIGSYVKNFLLIDTGVYAHGHSLRLPYFAKIAPDGPACGRLLPVFVIPPACKDVPAFVAAHADPRRFHFHAPPTYLASPREIRVLHSLGGDYVSFFERKASRNALEHFGRRETLTEVLGRYNVQPDAGGTVEGFASELLGRIVACIETHFPEHAGEYQAVSVRRAVSKDDWVLLQLVPVRGTLQQSLSCLRFKHGRASRATARTFVALSVGANNRLCVSLCQQCFAAKCDSNRLHTLFTIDAGTPCSPSVPCSTSQPSS